European Patent Application EP 4 535 003 A1, published April 9, 2025. Title: PREPARATION METHOD OF SAMPLE SOLUTION CONTAINING NEUROGRANIN-RELATED PEPTIDE AND ANALYSIS METHOD OF NEUROGRANIN-RELATED PEPTIDE. Applicant: SHIMADZU CORPORATION. Application JP. The sequence listing filed with the application follows.

SEQUENCE LISTING (12 sequences)

SEQ ID NO: 1 - protein, 26 aa, Homo sapiens
ERGRKGPGPGGPGGAGVARGGAGGGP

SEQ ID NO: 2 - protein, 29 aa, Homo sapiens
ERGRKGPGPGGPGGAGVARGGAGGGPSGD

SEQ ID NO: 3 - protein, 97 aa, synthetic construct
GSSHHHHHHSSGLVPRGSHMGSMDCCTENACSKPDDDILDIPLDDPGANAAAAKIQASFRGHMARKKIKSGERGRKGPGPGGPGGAGVARGGAGGGP

SEQ ID NO: 4 - protein, 100 aa, synthetic construct
GSSHHHHHHSSGLVPRGSHMGSMDCCTENACSKPDDDILDIPLDDPGANAAAAKIQASFRGHMARKKIKSGERGRKGPGPGGPGGAGVARGGAGGGPSGD

SEQ ID NO: 5 - protein, 31 aa, Homo sapiens
SGERGRKGPGPGGPGGAGVARGGAGGGPSGD

SEQ ID NO: 6 - protein, 33 aa, Homo sapiens
IKSGERGRKGPGPGGPGGAGVARGGAGGGPSGD

SEQ ID NO: 7 - protein, 34 aa, Homo sapiens
KIKSGERGRKGPGPGGPGGAGVARGGAGGGPSGD

SEQ ID NO: 8 - protein, 35 aa, Homo sapiens
KKIKSGERGRKGPGPGGPGGAGVARGGAGGGPSGD

SEQ ID NO: 9 - protein, 40 aa, Homo sapiens
GHMARKKIKSGERGRKGPGPGGPGGAGVARGGAGGGPSGD

SEQ ID NO: 10 - protein, 46 aa, Homo sapiens
IQASFRGHMARKKIKSGERGRKGPGPGGPGGAGVARGGAGGGPSGD

SEQ ID NO: 11 - protein, 24 aa, Homo sapiens
KIKSGERGRKGPGPGGPGGAGVAR

SEQ ID NO: 12 - protein, 25 aa, Homo sapiens
KKIKSGERGRKGPGPGGPGGAGVAR